European Patent Application EP 4 715 053 A1, published March 25, 2026. Title: 靶向血管紧张素原的核酸及其用途. Applicant: 施能康医药科技（苏州）有限公司. The sequence listing filed with the application follows.

SEQUENCE LISTING (53 sequences)

SEQ ID NO: 1 - RNA, 21 nt, synthetic construct
  source 1..21: mol_type = other RNA
ccacgctctctggacttcaca

SEQ ID NO: 2 - RNA, 21 nt, synthetic construct
  source 1..21: mol_type = other RNA
tggacaacagcacctcagtgt

SEQ ID NO: 3 - RNA, 21 nt, synthetic construct
  source 1..21: mol_type = other RNA
gtctcactttccagcaaaact

SEQ ID NO: 4 - RNA, 21 nt, synthetic construct
  source 1..21: mol_type = other RNA
cctcaactggatgaagaaact

SEQ ID NO: 5 - RNA, 21 nt, synthetic construct
  source 1..21: mol_type = other RNA
ttcctgtttgctgtgtatgat

SEQ ID NO: 6 - RNA, 21 nt, synthetic construct
  source 1..21: mol_type = other RNA
gctgggtttattttagagaat

SEQ ID NO: 7 - RNA, 21 nt, synthetic construct
  source 1..21: mol_type = other RNA
ctgggtttattttagagaatg

SEQ ID NO: 8 - RNA, 21 nt, synthetic construct
  source 1..21: mol_type = other RNA
ccaaccgaccagcttgtttgt

SEQ ID NO: 9 - RNA, 21 nt, synthetic construct
  source 1..21: mol_type = other RNA
ccgaccagcttgtttgtgaaa

SEQ ID NO: 10 - RNA, 21 nt, synthetic construct
  source 1..21: mol_type = other RNA
gaccagcttgtttgtgaaaca

SEQ ID NO: 11 - RNA, 21 nt, synthetic construct
  source 1..21: mol_type = other RNA
gaccagcttgtttgtgaaaca

SEQ ID NO: 12 - RNA, 21 nt, synthetic construct
  source 1..21: mol_type = other RNA
ccagcttgtttgtgaaacaaa

SEQ ID NO: 13 - RNA, 21 nt, synthetic construct
  source 1..21: mol_type = other RNA
gcttgtttgtgaaacaaaaaa

SEQ ID NO: 14 - RNA, 21 nt, synthetic construct
  source 1..21: mol_type = other RNA
gtttgtgaaacaaaaaagtgt

SEQ ID NO: 15 - RNA, 21 nt, synthetic construct
  source 1..21: mol_type = other RNA
caaaaaagtgttcccttttca

SEQ ID NO: 16 - RNA, 21 nt, synthetic construct
  source 1..21: mol_type = other RNA
cccttttcaagttgagaacaa

SEQ ID NO: 17 - RNA, 21 nt, synthetic construct
  source 1..21: mol_type = other RNA
gagaacaaaaattgggtttta

SEQ ID NO: 18 - RNA, 21 nt, synthetic construct
  source 1..21: mol_type = other RNA
gaacaaaaattgggttttaaa

SEQ ID NO: 19 - RNA, 21 nt, synthetic construct
  source 1..21: mol_type = other RNA
gcattgccttcggtttgtatt

SEQ ID NO: 20 - RNA, 21 nt, synthetic construct
  source 1..21: mol_type = other RNA
cattgccttcggtttgtattt

SEQ ID NO: 21 - RNA, 21 nt, synthetic construct
  source 1..21: mol_type = other RNA
ccttcggtttgtatttagtgt

SEQ ID NO: 22 - RNA, 21 nt, synthetic construct
  source 1..21: mol_type = other RNA
ggtttgtatttagtgtcttga

SEQ ID NO: 23 - RNA, 21 nt, synthetic construct
  source 1..21: mol_type = other RNA
gtatttagtgtcttgaatgta

SEQ ID NO: 24 - RNA, 21 nt, synthetic construct
  source 1..21: mol_type = other RNA
gtgtcttgaatgtaagaacat

SEQ ID NO: 25 - RNA, 21 nt, synthetic construct
  source 1..21: mol_type = other RNA
gtcttgaatgtaagaacatga

SEQ ID NO: 26 - RNA, 21 nt, synthetic construct
  source 1..21: mol_type = other RNA
ccatagctggttatttctcct

SEQ ID NO: 27 - RNA, 23 nt, synthetic construct
  source 1..23: mol_type = other RNA
tgtgaagtccagagagcgtggga

SEQ ID NO: 28 - RNA, 23 nt, synthetic construct
  source 1..23: mol_type = other RNA
acactgaggtgctgttgtccatt

SEQ ID NO: 29 - RNA, 23 nt, synthetic construct
  source 1..23: mol_type = other RNA
agttttgctggaaagtgagactt

SEQ ID NO: 30 - RNA, 23 nt, synthetic construct
  source 1..23: mol_type = other RNA
agtttcttcatccagttgaggga

SEQ ID NO: 31 - RNA, 23 nt, synthetic construct
  source 1..23: mol_type = other RNA
atcatacacagcaaacaggaatg

SEQ ID NO: 32 - RNA, 23 nt, synthetic construct
  source 1..23: mol_type = other RNA
attctctaaaataaacccagctt

SEQ ID NO: 33 - RNA, 23 nt, synthetic construct
  source 1..23: mol_type = other RNA
cattctctaaaataaacccagtt

SEQ ID NO: 34 - RNA, 23 nt, synthetic construct
  source 1..23: mol_type = other RNA
acaaacaagctggtcggttggaa

SEQ ID NO: 35 - RNA, 23 nt, synthetic construct
  source 1..23: mol_type = other RNA
tttcacaaacaagctggtcggtt

SEQ ID NO: 36 - RNA, 23 nt, synthetic construct
  source 1..23: mol_type = other RNA
tgtttcacaaacaagctggtcgg

SEQ ID NO: 37 - RNA, 23 nt, synthetic construct
  source 1..23: mol_type = other RNA
tgtttcacaaacaagctggtctt

SEQ ID NO: 38 - RNA, 23 nt, synthetic construct
  source 1..23: mol_type = other RNA
tttgtttcacaaacaagctggtc

SEQ ID NO: 39 - RNA, 23 nt, synthetic construct
  source 1..23: mol_type = other RNA
ttttttgtttcacaaacaagctg

SEQ ID NO: 40 - RNA, 23 nt, synthetic construct
  source 1..23: mol_type = other RNA
acacttttttgtttcacaaacaa

SEQ ID NO: 41 - RNA, 23 nt, synthetic construct
  source 1..23: mol_type = other RNA
tgaaaagggaacacttttttgtt

SEQ ID NO: 42 - RNA, 23 nt, synthetic construct
  source 1..23: mol_type = other RNA
ttgttctcaacttgaaaagggtt

SEQ ID NO: 43 - RNA, 23 nt, synthetic construct
  source 1..23: mol_type = other RNA
taaaacccaatttttgttctcaa

SEQ ID NO: 44 - RNA, 23 nt, synthetic construct
  source 1..23: mol_type = other RNA
tttaaaacccaatttttgttctc

SEQ ID NO: 45 - RNA, 23 nt, synthetic construct
  source 1..23: mol_type = other RNA
aatacaaaccgaaggcaatgcaa

SEQ ID NO: 46 - RNA, 23 nt, synthetic construct
  source 1..23: mol_type = other RNA
aaatacaaaccgaaggcaatgca

SEQ ID NO: 47 - RNA, 23 nt, synthetic construct
  source 1..23: mol_type = other RNA
acactaaatacaaaccgaaggca

SEQ ID NO: 48 - RNA, 23 nt, synthetic construct
  source 1..23: mol_type = other RNA
tcaagacactaaatacaaaccga

SEQ ID NO: 49 - RNA, 23 nt, synthetic construct
  source 1..23: mol_type = other RNA
tacattcaagacactaaatactt

SEQ ID NO: 50 - RNA, 23 nt, synthetic construct
  source 1..23: mol_type = other RNA
atgttcttacattcaagacactt

SEQ ID NO: 51 - RNA, 23 nt, synthetic construct
  source 1..23: mol_type = other RNA
tcatgttcttacattcaagacac

SEQ ID NO: 52 - RNA, 23 nt, synthetic construct
  source 1..23: mol_type = other RNA
aggagaaataaccagctatggtt

SEQ ID NO: 53 - DNA, 2148 bp, synthetic construct
  source 1..2148: mol_type = other DNA
agaaagtagaccctcaccaggcatggaatctgccagtgccttgatcttggacttccagcttccagaactggtatgcggaagcgagcaccccagtctgagatggctcctgccggtgtgagcctgagggccaccatcctctgcctcctggcctgggctggcctggctgcaggtgaccgggtgtacatacaccccttccacctcgtcatccacaatgagagtacctgtgagcagctggcaaaggccaatgccgggaagcccaaagaccccaccttcatacctgctccaattcaggccaagacatcccctgtggatgaaaaggccctacaggaccagctggtgctagtcgctgcaaaacttgacaccgaagacaagttgagggccgcaatggtcgggatgctggccaacttcttgggcttccgtatatatggcatgcacagtgagctatggggcgtggtccatggggccaccgtcctctccccaacggctgtctttggcaccctggcctctctctatctgggagccttggaccacacagctgacaggctacaggcaatcctgggtgttccttggaaggacaagaactgcacctcccggctggatgcgcacaaggtcctgtctgccctgcaggctgtacagggcctgctagtggcccagggcagggctgatagccaggcccagctgctgctgtccacggtggtgggcgtgttcacagccccaggcctgcacctgaagcagccgtttgtgcagggcctggctctctatacccctgtggtcctcccacgctctctggacttcacagaactggatgttgctgctgagaagattgacaggttcatgcaggctgtgacaggatggaagactggctgctccctgatgggagccagtgtggacagcaccctggctttcaacacctacgtccacttccaagggaagatgaagggcttctccctgctggccgagccccaggagttctgggtggacaacagcacctcagtgtctgttcccatgctctctggcatgggcaccttccagcactggagtgacatccaggacaacttctcggtgactcaagtgcccttcactgagagcgcctgcctgctgctgatccagcctcactatgcctctgacctggacaaggtggagggtctcactttccagcaaaactccctcaactggatgaagaaactatctccccggaccatccacctgaccatgccccaactggtgctgcaaggatcttatgacctgcaggacctgctcgcccaggctgagctgcccgccattctgcacaccgagctgaacctgcaaaaattgagcaatgaccgcatcagggtgggggaggtgctgaacagcattttttttgagcttgaagcggatgagagagagcccacagagtctacccaacagcttaacaagcctgaggtcttggaggtgaccctgaaccgcccattcctgtttgctgtgtatgatcaaagcgccactgccctgcacttcctgggccgcgtggccaacccgctgagcacagcatgaggccagggccccagaacacagtgcctggcaaggcctctgcccctggcctttgaggcaaaggccagcagcagataacaaccccggacaaatcagcgatgtgtcacccccagtctcccaccttttcttctaatgagtcgactttgagctggaaagcagccgtttctccttggtctaagtgtgctgcatggagtgagcagtagaagcctgcagcggcacaaatgcacctcccagtttgctgggtttattttagagaatgggggtggggaggcaagaaccagtgtttagcgcgggactactgttccaaaaagaattccaaccgaccagcttgtttgtgaaacaaaaaagtgttcccttttcaagttgagaacaaaaattgggttttaaaattaaagtatacatttttgcattgccttcggtttgtatttagtgtcttgaatgtaagaacatgacctccgtgtagtgtctgtaataccttagttttttccacagatgcttgtgatttttgaacaatacgtgaaagatgcaagcacctgaatttctgtttgaatgcggaaccatagctggttatttctcccttgtgttagtaataaacgtcttgccacaataagcctccaaaaa